European Patent Specification EP 4 045 009 B1, published September 9, 2026. Title: METHODS FOR TREATING BREAST CANCER. Applicant: Dinarello, Charles A. Tengesdal, Isak. The sequence listing filed with the application follows.

SEQUENCE LISTING (6 sequences)

SEQ ID NO: 1 - DNA, 24 bp, Artificial Sequence
  synthetic
tactctcaatcctatccctggctg

SEQ ID NO: 2 - DNA, 24 bp, Artificial Sequence
  synthetic
tgtgaggtttgattcaggcagatg

SEQ ID NO: 3 - DNA, 20 bp, Artificial Sequence
  synthetic
tgacgtcacggggtgatgtc

SEQ ID NO: 4 - DNA, 20 bp, Artificial Sequence
  synthetic
gaggatgcacccggaagtga

SEQ ID NO: 5 - DNA, 21 bp, Artificial Sequence
  synthetic
gctccaaaggacttgtacgtg

SEQ ID NO: 6 - DNA, 21 bp, Artificial Sequence
  synthetic
tgatctgaagggcagcatttc